European Patent Application EP 4 273 268 A9, published October 30, 2024. Title: GENETIC MARKERS AND USES THEREFOR. Applicant: Livestock Improvement Corporation Limited. Application EP EP23186997.5, filed July 21, 2023. The sequence listing filed with the application follows.

SEQUENCE LISTING (8 sequences)

SEQ ID NO: 1 - DNA, 20 bp, synthetic construct
  source 1..20: mol_type = other DNA
cctattttctggccaatgga

SEQ ID NO: 2 - DNA, 19 bp, synthetic construct
  source 1..19: mol_type = other DNA
cagcccaactggagtctgc

SEQ ID NO: 3 - DNA, 39 bp, Bos taurus
  source 1..39: mol_type = genomic DNA
gaccaaacagaccaacatgtttaaaagcctcaaaaacca

SEQ ID NO: 4 - DNA, 2387 bp, Bos taurus
  source 1..2387: mol_type = genomic DNA
ggcaaatgctgaggatactttccaagtgaaccctgagtgaacctctaatatatttatttcctgtggaaagaggaaggagccaacatgaaggaaaatgcagcatctagagtggttttcattttgctactttttctcagtgtcagccttctgaatggacagtcacctcctgaaaaacccaagctcgttaaatgtcggtctcctggaaaggaaacattcacctgctggtgggagcctggggcagatggaggacttcctaccaattacacgctgacttaccacaaggaaggagaaacactcatccatgaatgtccagactacaaaaccgggggccccaactcctgctactttagcaagaagcacacctccatatggaagatgtacgtcatcacagtaaacgccatcaaccagatgggaatcagttcctcggatccactttatgtgcacgtgacttacatagttgaaccagagcctcctgcaaacctgactttggaattaaaacatccagaagatagaaaaccatatctatggataaaatggtctccacccaccatgactgatgtaaaatctggttggttcattatccagtacgaaattcgattaaaacctgagaaagcaactgattgggagactcattttactctgaagcaaactcagcttaagattttcaacttatatccaggacaaaaataccttgtgcagattcgctgcaagccagaccatggatactggagtgagtggagcccagagagctccatccagatacctaatgacttcccagtgaaggacacaagcatgtggatctttgtggccatcctttctgctgtcatctgtttgattatggtctgggcagtggctttgaagggctatagcatggtgacctgcatcctcccaccagttccagggccaaaaataaaaggatttgatgttcatctgctggagaagggcaagtccgaagaacttctgcgagctctggaaagccaagacttcccccccacttctgactgcgaggacttgctgatggagttcatagaggtagatgactgtgaggaccagcagctgatgccacgcccctccaaagaacacacggagcaaggcgtgaagcccatgcacctggatcttgacagtgactctggccggggcagctgcgacagcccttcgctcttgtctgaaaagtgtgatgaacctcaggcccatccctccaagttccatactcccgagggccctgagaagctggagaatccggaaacaaaccttacatgtctccaggcccctcagagcacaagcgtggaaggcaaaatcccctattttctggccaatggacccaaatcttccacatggcctttcccgcagccccccagcctatacagccccagatattcttaccacaacattgctgacgtgtgtgagctggccctgggcatggccggcaccacagccacttcgctggaccaaacagaccaacatgctttaaaagcctcaaaaaccattgaaactggcagggaaggaaaggcaaccaagcagagggagtcagaaggctgcagttccaagcctgaccaagacacggtgtggccacgaccccaagacaaaacccccttgatctctgctaaacccttggaatacgtggagatccacaaggtcagccaagatggagtgctggctctgttcccaaaacaaaacgagaagtttggcgcccctgaagccagcaaggagtactcaaaggtgtcccgggtgacagatagcaacatcctggtattggtgccggatccgcaagcgcaaaacctgactctgttagaagaaccagccaagaaggccccgccagccctgccatagaatccagccaaggccgacctggctatctcccccacaaccccaggcaactgcagactccagttgggctggggactgggtcccgcaggttttatgcactcttgcagtgagagttatggaaggatgggttcaattgtgattttccttcagggaacactacagagtacgtgaaatgcactctaccagagagggctcaagaacagggttagaatgacactacccaactcccagttcactcttaattctctattttcaaccagttgcctctttgtccaacagctgattccagaacaaatcgttccatcttgtgtgatttgtagatttacttttttgctattagttgtcagattatatgttcaaagatataaaagcacattgcctagtattcttaagagacagtgccaataggtatataatctggaaaaggccttcatggtttcgtatgtgacagaggggtataagtcagtcaaaattgtttaccatgggaagatggtagataggagagaaatgccatgaaaaccactttgaagaccagttgcttaacctttgcactcctcttt

SEQ ID NO: 5 - protein, 581 aa, Bos taurus
MKENAASRVVFILLLFLSVSLLNGQSPPEKPKLVKCRSPGKETFTCWWEPGADGGLPTNYTLTYHKEGETLIHECPDYKTGGPNSCYFSKKHTSIWKMYVITVNAINQMGISSSDPLYVHVTYIVEPEPPANLTLELKHPEDRKPYLWIKWSPPTMTDVKSGWFIIQYEIRLKPEKATDWETHFTLKQTQLKIFNLYPGQKYLVQIRCKPDHGYWSEWSPESSIQIPNDFPVKDTSMWIFVAILSAVICLIMVWAVALKGYSMVTCILPPVPGPKIKGFDVHLLEKGKSEELLRALESQDFPPTSDCEDLLMEFIEVDDCEDQQLMPRPSKEHTEQGVKPMHLDLDSDSGRGSCDSPSLLSEKCDEPQAHPSKFHTPEGPEKLENPETNLTCLQAPQSTSVEGKIPYFLANGPKSSTWPFPQPPSLYSPRYSYHNIADVCELALGMAGTTATSLDQTDQHALKASKTIETGREGKATKQRESEGCSSKPDQDTVWPRPQDKTPLISAKPLEYVEIHKVSQDGVLALFPKQNEKFGAPEASKEYSKVSRVTDSNILVLVPDPQAQNLTLLEEPAKKAPPALP

SEQ ID NO: 6 - DNA, 2386 bp, Bos taurus
  source 1..2386: mol_type = genomic DNA
ggcaaatgctgaggatactttccaagtgaaccctgagtgaacctctaatatatttatttcctgtggaaagaggaaggagccaacatgaaggaaaatgcagcatctagagtggttttcattttgctactttttctcagtgtcagccttctgaatggacagtcacctcctgaaaaacccaagctcgttaaatgtcggtctcctggaaaggaaacattcacctgctggtgggagcctggggcagatggaggacttcctaccaattacacgctgacttaccacaaggaaggagaaacactcatccatgaatgtccagactacaaaaccgggggccccaactcctgctactttagcaagaagcacacctccatatggaagatgtacgtcatcacagtaaacgccatcaaccagatgggaatcagttcctcggatccactttatgtgcacgtgacttacatagttgaaccagagcctcctgcaaacctgactttggaattaaaacatccagaagatagaaaaccatatctatggataaaatggtctccacccaccatgactgatgtaaaatctggttggttcattatccagtacgaaattcgattaaaacctgagaaagcaactgattgggagactcattttactctgaagcaaactcagcttaagattttcaacttatatccaggacaaaaataccttgtgcagattcgctgcaagccagaccatggatactggagtgagtggagcccagagagctccatccagatacctaatgacttcccagtgaaggacacaagcatgtggatctttgtggccatcctttctgctgtcatctgtttgattatggtctgggcagtggctttgaagggctatagcatggtgacctgcatcctcccaccagttccagggccaaaaataaaaggatttgatgttcatctgctggagaagggcaagtccgaagaacttctgcgagctctggaaagccaagacttcccccccacttctgactgcgaggacttgctgatggagttcatagaggtagatgactgtgaggaccagcagctgatgccacgcccctccaaagaacacacggagcaaggcgtgaagcccatgcacctggatcttgacagtgactctggccggggcagctgcgacagcccttcgctcttgtctgaaaagtgtgatgaacctcaggcccatccctccaagttccatactcccgagggccctgagaagctggagaatccggaaacaaaccttacatgtctccaggcccctcagagcacaagcgtggaaggcaaaatcccctattttctggccaatggacccaaatcttccacatggcctttcccgcagccccccagcctatacagccccagatattcttaccacaacattgctgacgtgtgtgagctggccctgggcatggccggcaccacagccacttcgctggaccaaacagaccaacatgtttaaaagcctcaaaaaccattgaaactggcagggaaggaaaggcaaccaagcagagggagtcagaaggctgcagttccaagcctgaccaagacacggtgtggccacgaccccaagacaaaacccccttgatctctgctaaacccttggaatacgtggagatccacaaggtcagccaagatggagtgctggctctgttcccaaaacaaaacgagaagtttggcgcccctgaagccagcaaggagtactcaaaggtgtcccgggtgacagatagcaacatcctggtattggtgccggatccgcaagcgcaaaacctgactctgttagaagaaccagccaagaaggccccgccagccctgccatagaatccagccaaggccgacctggctatctcccccacaaccccaggcaactgcagactccagttgggctggggactgggtcccgcaggttttatgcactcttgcagtgagagttatggaaggatgggttcaattgtgattttccttcagggaacactacagagtacgtgaaatgcactctaccagagagggctcaagaacagggttagaatgacactacccaactcccagttcactcttaattctctattttcaaccagttgcctctttgtccaacagctgattccagaacaaatcgttccatcttgtgtgatttgtagatttacttttttgctattagttgtcagattatatgttcaaagatataaaagcacattgcctagtattcttaagagacagtgccaataggtatataatctggaaaaggccttcatggtttcgtatgtgacagaggggtataagtcagtcaaaattgtttaccatgggaagatggtagataggagagaaatgccatgaaaaccactttgaagaccagttgcttaacctttgcactcctcttt

SEQ ID NO: 7 - protein, 461 aa, Bos taurus
MKENAASRVVFILLLFLSVSLLNGQSPPEKPKLVKCRSPGKETFTCWWEPGADGGLPTNYTLTYHKEGETLIHECPDYKTGGPNSCYFSKKHTSIWKMYVITVNAINQMGISSSDPLYVHVTYIVEPEPPANLTLELKHPEDRKPYLWIKWSPPTMTDVKSGWFIIQYEIRLKPEKATDWETHFTLKQTQLKIFNLYPGQKYLVQIRCKPDHGYWSEWSPESSIQIPNDFPVKDTSMWIFVAILSAVICLIMVWAVALKGYSMVTCILPPVPGPKIKGFDVHLLEKGKSEELLRALESQDFPPTSDCEDLLMEFIEVDDCEDQQLMPRPSKEHTEQGVKPMHLDLDSDSGRGSCDSPSLLSEKCDEPQAHPSKFHTPEGPEKLENPETNLTCLQAPQSTSVEGKIPYFLANGPKSSTWPFPQPPSLYSPRYSYHNIADVCELALGMAGTTATSLDQTDQHV

SEQ ID NO: 8 - DNA, 2389 bp, Bos taurus
  source 1..2389: mol_type = genomic DNA
cgggcaaatgctgaggatactttccaagtgaaccctgagtgaacctctaatatatttatttcctgtggaaagaggaaggagccaacatgaaggaaaatgcagcatctagagtggttttcattttgctactttttctcagtgtcagccttctgaatggacagtcacctcctgaaaaacccaagctcgttaaatgtcggtctcctggaaaggaaacattcacctgctggtgggagcctggggcagatggaggacttcctaccaattacacgctgacttaccacaaggaaggagaaacactcatccatgaatgtccagactacaaaaccgggggccccaactcctgctactttagcaagaagcacacctccatatggaagatgtacgtcatcacagtaaacgccatcaaccagatgggaatcagttcctcggatccactttatgtgcacgtgacttacatagttgaaccagagcctcctgcaaacctgactttggaattaaaacatccagaagatagaaaaccatatctatggataaaatggtctccacccaccatgactgatgtaaaatctggttggttcattatccagtacgaaattcgattaaaacctgagaaagcaactgattgggagactcattttactctgaagcaaactcagcttaagattttcaacttatatccaggacaaaaataccttgtgcagattcgctgcaagccagaccatggatactggagtgagtggagcccagagagctccatccagatacctaatgacttcccagtgaaggacacaagcatgtggatctttgtggccatcctttctgctgtcatctgtttgattatggtctgggcagtggctttgaagggctatagcatggtgacctgcatcctcccaccagttccagggccaaaaataaaaggatttgatgttcatctgctggagaagggcaagtccgaagaacttctgcgagctctggaaagccaagacttcccccccacttctgactgcgaggacttgctgatggagttcatagaggtagatgactgtgaggaccagcagctgatgccacgcccctccaaagaacacacggagcaaggcgtgaagcccatgcacctggatcttgacagtgactctggccggggcagctgcgacagcccttcgctcttgtctgaaaagtgtgatgaacctcaggcccatccctccaagttccatactcccgagggccctgagaagctggagaatccggaaacaaaccttacatgtctccaggcccctcagagcacaagcgtggaaggcaaaatcccctattttctggccaatggacccaaatcttccacatggcctttcccgcagccccccagcctatacagccccagatattcttaccacaacattgctgacgtgtgtgagctggccctgggcatggccggcaccacagccacttcgctggaccaaacagaccaacatgctttaaaagcctcaaaaaccattgaaactggcagggaaggaaaggcaaccaagcagagggagtcagaaggctgcagttccaagcctgaccaagacacggtgtggccacgaccccaagacaaaacccccttgatctctgctaaacccttggaatacgtggagatccacaaggtcagccaagatggagtgctggctctgttcccaaaacaaaacgagaagtttggcgcccctgaagccagcaaggagtactcaaaggtgtcccgggtgacagatagcaacatcctggtattggtgccggatccgcaagcgcaaaacctgactctgttagaagaaccagccaagaaggccccgccagccctgccatagaatccagccaaggccgacctggctatctcccccacaaccccaggcaactgcagactccagttgggctggggactgggtcccgcaggttttatgcactcttgcagtgagagttatggaaggatgggttcaattgtgattttccttcagggaacactacagagtacgtgaaatgcactctaccagagagggctcaagaacagggttagaatgacactacccaactcccagttcactcttaattctctattttcaaccagttgcctctttgtccaacagctgattccagaacaaatcgttccatcttgtgtgatttgtagatttacttttttgctattagttgtcagattatatgttcaaagatataaaagcacattgcctagtattcttaagagacagtgccaataggtatataatctggaaaaggccttcatggtttcgtatgtgacagaggggtataagtcagtcaaaattgtttaccatgggaagatggtagataggagagaaatgccatgaaaaccactttgaagaccagttgcttaacctttgcactcctcttt